European Patent Application EP 4 299 724 A1, published January 3, 2024. Title: Novel bacteriophage having a specific bactericidal activity against Clostridium perfringens and antibacterial composition comprising the same. Applicant: CJ CheilJedang Corporation. The sequence listing filed with the application follows.

SEQUENCE LISTING (1 sequence)

SEQ ID NO: 1 - DNA, 51423 bp, bacteriophage CJ_CP_20-11-1
tatatatatattacatggtgattacatcaatggcaggctattgccttgcctccattatcattacggcaggcatatccatgcttccgagcttttgccctatatagaaaaacccagacggtcagcgatcgagctcttgattttgttttgtcgagggagagaacagtaagagagaacccccgaacgttgacagttgtacttacttctcttataatgacagtaaaggagggataaccatgaaaacattatttactgatacaaaactagtattaattgaaactactaacttcttcattatgttacaagaagaaggtaagtatgtactatctaaaacaatcgataaggagatgggagaacaaatacacagagtatctaagttagctgcccttgtatatactaatgaggagtatactaactctaatgaaccaagatctatatacttagatgacaatttcttatacgaagtgcttggtaatgggaagtatattataagatacagtatataagagcccacaatcaattctaaggccttttagatatgtggtaatgtgattttacttataatgtggtagagacaccttacaggagctgctagaggcctttaaaggaggtatatcatgtatttatgtaatggtaaaatagtcaagaataaaaatgacttaaaagataagtttggtggtaaatcagtagtattcatcgatggggatgtagctacagtaatggactttagtgacagaaagccaaagataacaaaatatcttattagggaggtatcacatgataaacacatcattattgaagagactggaagggatagaggaaaagcataagcaaaatactgatgagataagaaagaacctaaactatgccagatatttgattgagaaacagtattgtcatttaacaaaagaacagaagataaaattgggacagttcttaggattgactgagaagaagttaaaagaaatacaagagataaataatcagttaataaatttgagagtggggctaagttatgaagtcgtatgtaataaccagaaaaaatagtggggtatctttagcagatacagacatgggacaagtattagctaagatactatgtaagcatgggggaacacttaccattgaggaaattgaaccagaacatattggtcaaactttttctattgtagaaggtaaaagaatatggtataatagaaaaggaggtgataatattggggagaagaagtgctatgttaattctcaagtatgactgcgaagaaactccagaaaggattgaattacgaaagaagtggttacagatttgtcttcattcaataatatattatagatatgacaacaatatctggacagaccaacaatgggatgagactgccagagaggtagttaaacttaagaatgagaatccaggtttagtaaacagtatgccatttaggaatgaccttaaagtctttgatggatccactggctttaacctttcatgtatgcaagatattaagatgttaaggtgggctcaaaacttacttgactttcatgttaaacgaggacttgatggaaagagtaagaaaaagaagaagaagaggaggaaaaagaaatgaacctacttgagcactatataaaaaaggtacacagtgtaagagagtaccatgaatttgataatgaaccttgggctaaaggtaaacaatatgtagaagtagacatggactatatttgttattctaatacaccacaaagagtgaagatggtatttactgttgatgagtgggagaagataaaatatagaggctactacatgggataggaggaatagttatgataagagaaatgggcatgagaatgctaataccagaaatacatgatataaaagatagggatatacaaaattttgtaagaaaggccctaaatgagatagttgatgaaaagttctttataatacctgcaagtagtactgggaaatatcatccaacttatagtgcaggggtaggaggtttgttaagacatactaaagctgcttgttatataggtaaagcattatgcgaagctgagatgatatgttcaagggacagagatatgataatagctgctttaatattacatgacattaataagccagataaagaacatccatatatggttagagagacactatcacccctagaggaagagtttccaataatatacaaagtggtagttgaactaattgagtctcatcatggtcaatggggtagtgttcctattaatagttattcccagagaatagtacacttggctgattatatcagttcacagaaaggtttaatattctcatatgaccaaggaactgattattctgacctgttatgggaggagaagtaaatggtgctaggggtaataaccctagtatcaatatttttactaggagtgtttataggttttgaggtgaagaaatggaactaggttttgcgatactagctataatagtatcaatatttttagaaactaaatatataaaggagtagattattatgtcaagagcaagagctgcaaggagaagagccgaaagagagaacaaaaatcttaatgttcttaaagctgtggacatcatgttagccttatcatgctatacattaaagaaggaaggttatggtaagactagaatgactaggtttgtggaagggatgagtaaacacacagaggagattgaaaagggaacacttaactatgaaaccataatgggagagattaaggatttagtaccaccaggtatatttgatttaggggaggagtcaaaggagtgatagtattgggatatttattatgggcatttagaatattaggcatacttgtaatagtatggtgtataatggaggcgatcagttgtgagcaataagttatattttaggtatagtgctatgaactctggaaagactactcagttaatccaggtagcacataactatgaagaaaggggaatgaagccattagtagttaagcccggaattgatactaaaggtggaccatgtataatcagtagaataggggtagcaagaaaggtggatgttcttctacctcctagagttaaattatcaaaaatactttctgactttgagtctaattattgggcagtagatgttatattaattgatgaggtacaattcttatccagagaacaggttgatgatctgttaaatttatcattacattatcctattatatgttatggattgagaactgactttaaaagggaaggatttgaaggaagtaccagattattacaagtggcccataatattgaagaattaaagaacatttgtcaatgtggtaaaaaagccacattctcaatattaaaataccagggtaaatatactgaccagggtaaccagatacaaattgataaccagcccgaaagtgttgaatatgaagccgtttgtaatgaatgttataataaattaattttttctaaataactcgttgacaggctatataggatatgatattatagtattgtaatcaaattacaaacaccaaccaaaactttataattagttaatttcaaactatactaaatttgttatttaaaaattaaaaatatggaggaatgattattatggcaaaaggaaaagcaaaatggttagaggaagcaaacaataaggagctaattgtaatcgtacaatctgctttaaattctggagatgagaaagaagttaaaaaggctttaaaagctattgtggaattagatgaaagaactcctgacacagatggacaaataactgtagaggaagcattagaatcattagaaatggctgtaggaactgtaaaggctgcataccaagcagaaatagatgctgtggaagatgaaggtgtagtagatgctgacttcgaagaagttgatgaagacgaagcagaagaagaagatgaaaatgatttagaatcattatctaaaaaggaattagctgctatggctaaagacttaggtatcaaaggagctaagaaaaaagataaagatgagttaatcgctttaatcaaagaagctcaaggtgaagaagaagacgaagaggaagaagaagaggatgaaactcctgactactctgaaatgactaagaaagacttaattgctcttgctaaagaaagaggaataaaagttaataagaaaatgaaaccagctgagataattgaattattagaagctgatgatgaagaataattctcatcaaataataaggggagcaaacttgctcctcaaattttttacttattttagaaacagatgttagagggggatgtataaatggcaagaggtggaaattcaacttatactaaagcagtatattgttacaacaataatagggagtatagatccttcagatatgcagctaaacagttaggagtatcggctgttagtataatgagagtagttaacgggactaaaccacatatagggggattagtattcgctgagatagaggaaggcactagaaaattaaagccaagaggagaagtagttccatacttgaaagaattaggttgggataatatagacttataatagggggtataatatatggacataaagttcttgaaggatatattctctaaacaatgtgaaaatagagattacattatcctagcagctagaaaaggtaaagaatggaaagatgtaccaatcaaatataataagaataacattgacaaaaaactaaaggactttgaacaacagtataagggttatgatttatattggagcccaatgccctatagtaatcctcaaagaaggatagttaacttcatagagactaaatacttaatacaagatatagatgagcatactgacccattggggattaaacctaaaccaagttatctgtgggaaagttctcctggaaaatatcaggggctatgggaaatggataggtatatagaggctaatcaatatgacgaaataaatccagcattagctaaacatataggctgtgactcctgctttgatgttactcatgtatatagaataccaggaactattaactataaatacaagaataaaccaaaagtaaaaagacctatacacactaaggagatatataagcctaaggtgatcgctaaggctgttaaggctgtaagtaaatctaatgatagtgttaaggtcaatataggaggatctgaggcctcacaatctgaaagaaagatatatgctaaatataatataccaaagaaggttagagacttactggctttagatgacattacttctttagatagaagttctactatatggtatattgagaataaattacatgaaataggactagagcctaatgagattatattattagttaagggctcagcttttaataaatataagggaagaaaagatgaagaaacaaggttaagaaaagaattggataaaatcataggaggagaaatagaggctgatattgaaaaggctgaaagtactaaactgagaatagatagttatcaggatgttatgggtaataatggtgccttcccaggttggttagtacaaggtttctggggtagaagatctcatggaattgtggctggacaaccaaaggtatttaaatccacatttacacaggacttagctatatcagttgctagtggaagacccttcctaggtcaatatcctgttctagaaccaggcccagtaattgtagttcaaaatgagaatgctgactggattatgagggatagaactgaaaagataattagccacagaggagtagttggtaatgtggatataaagggtaagagaagacttaaagttaggtttgctccagatcttcctatcacttttattaatcaacagggatttatgttagatgaagaatcccatagaaaacagatagaagaattaattgatgagataaaacctgtactagtaatattcgacccattatatcttatgtttaggggagatcttaataatgcagctgatcttaatcctgtactacaatggtgtcttaaacttaagaatgagaagcatacaggagttatgttaatacaccactataataaaggtggaaatgccactcaaaccagaggtggtcaaaagatggctggttcattcatattacatggttgggtagaatcagcattatatttaaaaagacctgatgacttagaaggtgacgatgaggagattgaagtagatatagataaccttgataaacaaagccatttaccaagtaaaatcattatggatagagagttccgtcttgcaggacaattccctcaaattgaattgaatttatcaatgggagaatttggagatccatattatcatgtagaagtagcaatacccagaaaagaagtaattgtgaaacctgaggacaaagccaaagttatagaggctgtaaaatcaggagctcataccaaggaggagatagtgtcaatatcaggattaaattcacagaaggttaatccagttctagatactttaaaagatactattgtatattctccggataaaggttataatataagtaagaaactaaatattgggaggaaaaaggcatgataataaagtgtaagaggccagcaggtcataatcatataaaggcctttgtagtagtaattattgctagaggtaagaagaataaaatcacttatcattcaggattgaaatatttctatacctataaatcagctaaattatttatagacaaagttatggaagaatgtccctgggctgaattttattgggtggatgtccatgaagcccataagatccctgaaggcgaagagatacctaagaagaaaatgtggtgtccatattgtcaaactattcaagaatttaagagaagccaaggaggttacaagaattgccctatctgtggtataagtgaccaagacttttatgtaaaatgtatgaatataagatatagggaggctaaggctaatgcgaagaagaaacttgaaggaagtaatactaatcctagggatatcattgtcaatggggataatgctaactcagggggcaaaactaatagaaagtcatcaccaaagaaaaagtcaagaaaagttagtagaaaagcttcataatgctttagactataatgttattgagacttctccatctggactagatggggaggatcttattatcaaactaaaccttaatagtcctaaagaccttacccctaacaacttatctaagttagctaatgaggttatggtcaataacttaggagctcagaattatactatacttgtttatgatagtaatagaccagaaaatcttctggctgttatagatatacctaaaaattctaaaataacctttgacataataaattaattatggtaatataaaaatgtagaaggaggagaatttaatggtcaataaaaagtattacatcttgaaagaccttaatgatgacaaaccccaactatggaagggaagtttaaccactgctactaagatagcaggagcattaggagttagtgtgataaaactaaataggtatttagtaagaaagggatttgccagaaggtacaatgagcatacacttgagataatagacccaatccttgctaaagaacttggttattatgtaactccaagtaagtcccttataaatcctttatttgaatataatgataaaggagtacaatatatactaaacttaatagtagaagatctaaagaatggaggagagctttaatgattatcattttaggaatggataactcaggtaagaccacaacagctaagaacctaactaaacacagaggaggagaatatatccaatcaatgggacctggttcttatgaagaacaaagagaatgggtattaactcaaattgtgagaaaaggtgaaagggaagctatacatgatagatttacttgctttgaagaaatggtgtatggacctatcatcagagatagtagtaatttcaaccttgacagtaaggagctaaagatcttaaaacatctatgtaagccaactattgtatatgctagaccacctagggaagtgatcttcaattttggtgatagagaacagatgccaggagtaattgaaagagctgaacatctactggctagatatgatgaactgatatggaagttattctgtgatggatggaatgtactggtatatgattatactacttccaatgtggagaagctatcccagttaatagatgactcaagtgctaaagaagctataaaccaatttataaatatatcaagataagaggagagattgttatgaatataaaccatgcagtagaagaaaaaatagaaggagatagattacaagctatctttaatagacaaaaggagttaatggagaaatatcatcatatagaagctagatcaggattatgccaaactgaagactgtccagttaacttaaatgataaaagaggtcaagctagacttaaagattttgcttggagaatgactgaagaagtaggagaagcattggatgcttataatcatgaagaccattaccaagaagaattaattgatggattacacttcttaactgaatttacaattctagctggtaaggattataatactatagataataatgctatattagttgatagcctagagaacttatatcataaggctactacatcaccagaatttcctgaaatgttagtagaagaagctgtaactgacctggtaagagaaatgggtatgtgctgtaactgccttaagaataaaccttggaaacaaacttcaatgctaacagatgtaaatgcttttaatcaaagattattcaatgtatgggtatgttacattaaattattagctgtatctggcttagaggtagatgacatagtaaatatataccttaagaaatcacaggtaaataaattccgccaaagatctaattactaaaataaatacttaggagaaggtaatatgctaataagagactataatgattttgatgacttattcttaaaccttaatagggaaatgattaccaatccagaagaaactatgatgtatactcagaacatacagggctttcaggaggacttagttctctcctgtaagtcccataaatgtactttaaatctaggggactttggatataaagaaggtaagtggggacacctattaagatcatacattgattatccacaattaattgaatttagagaaaagcttaccaagataagtggtatgagctatacttattatttcaacaggaaaaaagctactaatggttcttgcttgatagctgcagtagtaactagaccaaaaagaaaaggaccttggaaacacttaaaaattatgtatagagtatgtgaattacaaaagaaattcgcagctgatctagtattaataaacaggttcattgaagaactacctcaagaagtatgtgagatagataatattacttttcatatgtctcaagcttatttgtcaggaatgtttataaatggatatttcaattattttaaggtaccaagaaagagtattgctaatagcaaacatccttggcataaatccttgaatagtaactataacaggttctttaaatcagaggaccagatacactcttataaagctctccagaagatgcagttattacattttggtctggagaaatttccaaagatagatatcaataaattatctattgacaagtactttaataagtagtataattaacttaacaaaattaaataaatggaggaattaaactatgagaatttatattaatgctcaagaagcatttgaagaagtaaaaagagatttatgtgaaatggggattggggtaagacccaaaactatgcaagataaagttatagaaggtaatccagattatttcacaaaggagttacaaaactatagttacacaattctagaaagtaaacctgaagaagttccaggtgtatctcaaccttgggcagatgctgaatttagagaaaggatctacgatccacaaggtgtcatcaatcaatactctcttgaagaaagagaagaattatttggtatacatccacatcatactagggaggctttcataaatcctggtaaagcttatcaattaagacctgaggtatggaatgaatatctaagagatggaaaatttgggtattcttacaatgaaagaatttggcaatacagacaaattgaggatatcatcaatagaattaaagaagatccaggctcaagacaattatggttatctctgtggaatccagctattgatccattcaatataggaggagtaactagagtaccatgttcattaggatataacttccaagtaagagaaggtaagctaaatatccattatgttatgagaagttctgattttgctactcactttgctaatgatgtttatcttgctatgaaactattacattgggtagctgaacaaactggctatgaaccaggaagtttctctcatacaattttctctcttcatgtttacaacaaagatattaagggggtattctaataaatgagttacatgagaaaagaaagatataaacattctgatcttaataataaggttaacaagaaggaaaccctaaagcaatttattaggaatactgaaaaggaatttgatttagaaccagctaaccttggggacatgactaggaatgaacttaataactatataaattatatggatgaactgtggagtaagtaatatgtataattatagtgatgataacagacctaagaacaataacaatggctgtcttggttgtttaattataatcttagcagctataggattatgggtaataatttttgatattgccaatataatatatcatatgatattctaaatttaaagggggctatcctaatgaaaaatataatttgtcctatgtgtaaaaactcagtaacattaaaaagaaaatatggagctatgttttggatcatgattttcttaactggaggcctatgggtagtaaccatacccttcaaaaaacataaggtctgtccagtatgtaactcaatcataaaataaagataagggcctttaggggtcctttctatttaggaggtaatattttaaatgagatgtaacaactgtaacctatatactcactcagctccctcatgtatagaaggaacttgtgtaggaaagaaaaagaagccaagaataatggtcataaatagtttagctaatgatagggatgaggccaatagaatagctactcctgataaatcattacttgataaaatggaaggtctagacttttattataccaatgctattaagtgtagaactcctaagggtactaaaatcaaagtatcagagattaagaaatgccaagaacatttacttaaggaaattgaaaaatataaacccgaatatgttatgatcttaggatctcaagcattaaagatgctaagtaatgaaggtataacttcaatatgtggagtacctaagaagcatgagaaatatggctttaagtttattgccagctattcacccggtgtagttgcatatgacccaactaaagcacaatttgtagatcaggcctttaataactttaaagccatggtaaaaggtaaagagcatgaattacctgatcttaacataaaacttattactagtatgaaagaactaaaccaggctttcaaatatttaagggatgagggttataatagagtatcatatgatatagaaactagaggcttagataggtttaataataacattactctatttggttttggtaatacccaagtacagtatatactgcctttagaagtcaaatatagcccattaaggggtaagcccatagcacaaagaagattagctaaatccttgattaaaagacttaattctgagatgaaggaaagaatagcccagaatggtaagtttgatgataatttcttaaaggagaaatatggtattaagccaatcataacctttgatactttactagcctcacattgtttagatgagaatactcctaatggtcttaaggagaatgctttattacattgtaatgctaaagactgggatataaataagaaattaaagactggaaatgtggagactaaatcagactttgaggattatgttaggtatctggggtatgatatatactatacatttgctctatataaaatatttaataaaagacttaaaagggatgagagcttatataaactattccaccacttatacatcccagctagtaaagcttatgaggatgttcagttcaagggtatatatgtaaatcaggagaaattcaaagaggttgaaaaatacttaagatctgaactagataagattgagactggacttaagaagtatactaatggccaggatattaactggagctcacctaaacaggttggagaatttttatatgatatacttggtcttcctgtgattgaggttactgactctggagcaccagctactggagaaagtgtattattaagactaagagataaacatccagcagtagaactactattacagcataggggagttcatatacaaatttcccactttatagatggttggctaaataggatgcacaatcatagattatatccaaactttaaacttcatggaactgtaacaggaagaacctcaagtaataatcctaatctacagcaagttcctagagataagaaaatcaggagtttattaggaccatctcctggaagagtattcattgaagccgatctatcccaggccgaacttagaatagctgctatgatggccgatgaggataatatgaagtttatttaccagactggtggagatatacatgactccacatataatattatatctggggaagatatcaatgatgagaaagatccagcagttaagaaggagaaaaggaaaaaggctaaggctgtaaactttggtttcttatatggtatgcaatggaaaaaattcaaggattatggaagagacaactatggtcttaaattaacagatgaggaagccaaaacatatagaaggaacttctttaataaataccctaaactattaacatggcatgataaacaaagaaaaattgttaaagccaatggtgaagtaagatctctaataggaagaattagaagattacccgatatatattcatctgatagatctaaagctgctgaagccgaaagacaatgtattaactcaccagttcaaggttttggttcagatatcactttattaggcctatgtgagattacaggctatgctaaatatgttaatcctgaatatgtattagataagtctaagtttgatgtattaggctcagtacatgactcaatattatttgaagtagataaagactatgtggaagaattagcttggaaagtaaaatcaatagttgaaaataataaagtattaaagaaagtatttaaatttaccccaacagtcccaataatcatggatatatcagttggttattcttggggaggatgtgttgaactggattttaaaggtgattggaaaagccagataagaaaagtgttgacagatgaataattatctgataatataaatattgtaatgaaaaggaggtataaggatgttaaaaataagtaattccagaattaacaaattcttgtcttgtccttatgcccattatgttaaatactatgaaggtctggtacctaaaagaagtggagctgccttacaaaggggctctgctatccaccaggctatagaagactaccataatgggaagagttggaaaaaatctgttgataaattttccaaagagttttacaaaaatacatttaaagaagagatccttgaatttggagatattccaaaaatggtttattctttatgtgataactatttccactattatgatgaaaaagaagataatgtaacctatgtggaaaatgaacatcacttcgaattaaaactatgtaagggtgtaactctagaaggctatattgatagtgtcttagatgtggatggaaagatatgggctaaggaaactaaaacctacaaaaagatgcctgatagaaatttcctgatcttcaatagacaatctgctatatatacctgggctcttctacatgaatacccaaaagtaagtggtactatatgggatataatattagctcagcaaccaggtagaccagaattaactcaaaaaggggtattatctcaaaagaggattaaatccacacccctagagttagaaagaggaataagagaattaggattagatcctaaagattatgagtcttatattaattctgctagatgggaagacttctttgtaagacacccaataatattatcaaagaatatacttaacagtgtaatgattgatactattgagatagctaaacttattagagatgagggccacaaaagaaaggaaaagaaccttggaaaaggttgctctttctgtgaatataaatctttatgccaagctgaacttttaaatcttgataaagaatttattattaaggctgactacaaacaaagggaggaaagtgacaatggcaaaaaagcaaaaatcaaaatcaaatagttttgaggacagattagtggatctatatgatatagatgagcccacaatactaacactttatggaagatctggttcaggtaaaactactatctcaggaacactacccaaaccaatattctttattgatgtaaaggacaaaggtactctatcagctagaaacaagcttagagttaaaagaggagatatacaagtatttagtctaaagagttttgatgacatatacgaggcttatgattacctatcagaaaacactgataaatttaaaacagtagttatagaccatttaactgctttacaagaattaggtaatgaaaaggtcaaagctgaagaaggtaaggaccagatgagccaaagaatgtttggaaatgtggctaattatatgaaagaggttataaacctttataaagaattaaatgaggaaggtatactaccatgctttatagtacaagataggttagaatctggtgatggtgaaggagaagaccaattaatgcctgaggtaggaccaggattaatgccatctgtatctaaatatttatgtgctgtatcaagagtaataggtcatacttatttatatgaacactcagaaaaagagggtatgaaggttaagaaagaaatccagtatagactaagactaggacctaacccttattatattactaaatttactagacctcaaggatctgaatgtccagcttatctggtacatgatttaaaatcaccaacaactatctgggaggatattgaaactattctggctggtgaatggaataataagccagctaaatctggtaaaaaaaccagtaagaaatctggtaaaaagaaaaaataaaattttctaaaaatacctttgacaaccaattaaaaatctgataatataaacttgtaaacaaagaggtacaatatcttgacaaatatttatctcataatgatattttaaaatttaaggaggacaataacatggctaaaaagactactaagagaggtaacaaaaacaaaggaggattaaagattgatctttcaaacgttgaaacttcagttactatcccagaaggaaattacattgtggaagtagaagatgtagaggttaaggtttctgaaaatagtggaagcaattatttatcatttacttttgtaatagcagaaggaaagatgaaaggacaaaagttataccacatttgctcacttcaaccacaagctttatttaacttaaaaggtgtgttagttgctttaggatttgatatccctgatgaggagttcgaattagatacagaagctctagttggtttacaatgtggggtagaagtatcacatgaaatatatgagggtaagaagaaatcaagaataactgattttataaaccttgacgaagctgactctgatgatgacgaagatgaggatgatgactcagatgatgatgaagaagatgatgaagaagaaaatgactatgagtcaatgactttaaaagaacttaaagctgaagctaaggacagaggcttaaaggttaaaaaaggaatgtctaaggatgacatcatagaaatgctagaagaagatgatgaagaataaaatttaattattaaaatatgagggcctttaaggtcctcctttatttacccttggaggctactattatgcttgaaagagatgtggttaaatccataatgaatatgcttaaaaaagaatacccaggtttttggtttaaaactcatgggggaccatttcaaatagctggcttacctgatatactaggttgccacaaaggtaagtttattggtattgaagttaaacttcctggaaaagaaaagaacctaactcaaaaacaaaaagacattataaataaaataaatctagcaggaggaatagcttttatggctacctcagctgaatatacaaggaggagattacatgaaaaatttagaaagacaccaacaattcctaggagaactaggagatctgtatgaattaaagaataatctatatggggataatttccacaagacttatcttgaatatggaaaccctgttctatgtataagacttgaagataagctaggaagagctaaaagtttattactaggagatcaagatgacttcccttcatatgctgctcaaaaagaatctgtggttgatactttactagacctagctaactatgccattatggctgctatggaactaactagtgatgataactcagaaatacatgatcttagtaaagaagaatatgatgaagaagacctagatgataatgacgatgatgacttagatgatgatgacaatgtttacgacgaagaagaattagattttgatagtatgaataaagaatccttaaaacaatatctaaaagataatggggttaaattccatagtaaggcctcaagagatgaacttgtaaaactggctaaggaggtataaggaggaggctttaatgcctcttcttttttagtatgaagagaaaattatttaaacatcagaaagaagcattacaactatttttaaataaagaaaagtttgccctatttatggacatgggtacgggtaagaccttagtccctattgtggcccttgagaaacttgaaggtctagatactgtactaatattctcacctaaatctattgtatttaactgggagtctgagatccataaatttactaaacttaaggaatataggatatttaaattacagggtaataagaccaaggttatggaaacctatagagctataaaatcctactcaggattaaagattattattgccaattttgagaaggctaggttgatggataaataccttatgaacttaaagccacagtttattgttgttgacgaatcccataaggtaaagaatagaaatgcccagatatctaaggctctatataaaattgctactaaatgtaaatataggttgataatgtcagggactcccactcctaatggttatgaagatttatttatgcaatataaaattatgaactcaaatattctaggagttaattggaaacagtttgaagatgactttataatcaaaggaggttatatgaactatgaaattgtggggtataagaatgaggaaatattaaagaaccttatgcaccagaattgctatatagtaagaatagaagattgtattgatttaccagaacaacttcctgatctgtatttaacctgtgaattaaatagtaaagccagaaaggcctataatgaccttagaaaggaaatgatagcacaactagatatagtacaggaaaacattcctagaaagcaattaaaggccttattaaggtctaatggtataccctatgagagtaatgagccctatgaggatttattcttaagggctaatatgtttatcaaccaattaacagctgatcttactattacccaatatttgaggctacagcagatctcaggaggatttatcacaaacaatgtaggaaataatattaatattgataaaggcaaattaggcttgttacaggactatctagaaggatataaaaagcctgttgttgtaatatgtaattttcttgaggaaataaaacttatacatgatacttttaaaaagacccacagagtagaatgcttaacaggatctactaagaatagagctgagatcaataaggattttcaggagggcaagattgatatattaatactacaaataagctcaggtagtgttggtctaaacctcttcagggcctcaaggttaatattctatagttggaactataaatatgatgattatgtgcaagctattgccagaatcaaaaggaatggtcaaaaggagccttggcaaataatacacttaataacggagaatactattgatgagaaaatattaaaatcaatacagcttaaaagggatagagcagaaaaactgttgactattgataagtaatgtggtaatatagaattgaggtgataagtaatgagaaaagaacaacctagaataagtaatcatactgaaatagctaaggctttaattgaggctggtaaaactattaaagctctaaccaagattaaagtcaaggaggaaaagaaaaaacaaaaaagacttgaaaggttaagactcctaaatgaggaaaagaagaaggagagagaattaatgaaagaatttaatcccgatgagcctaagaagccaagaaagaaaaaggacaaacctataaagaaggttgatctgaataaagttgaggctaagggaacttaccctacaccttctggaggtaatgcacctacgggaacagttgacttaaaaattttatgtgagtcattaggattagatccaagtaaagccagggccaagctaagaaagcaaggtgtaaacaaaccctataaatggtcaggatctgaacttgaggatattaagaaaatgttaaaataagggggaggtttaaaaacctcttctttttcgttgacaatatccacagtatatggtaatataaatattgtaatcaaacaaaaaaggagagaactgaatatgaaagatcttgaaaaacttacaagggaagaattgattgaacttgtaaaggagttatctattgattggacaggagcctataatagaaactataagattgaccttgatgagtatgagattgtatatattgatcttaatgatctaaaagagttcaatgataaattaggtcatctagaaggagatgtgtatatacaatacacggtaaatcttattaaggcccatttacatcctgagaaggatatattgattagagggggtggtgatgagtttgtagttatcagtgatatagcttataatctgtgcaataccttgaatatataccctgagctatcatgtggctatggtaaaggtaaaactattgaagaagctatagtacaggccgactcaatgatgtataagaataaaaaatctaagaagttaagatactcaaaggaggattagttattatgaggttattatggttaaaagaatatttggatatatgcaatatcttgggtattgagcccacaatggaatcttgtgctaggtggggaaagaataaaaaactatcagggttttcattaaccccagtgggagcaactaaatagttgcttctttttaaagcgatccgatacctagcaactttcatgccaaaaagaaattcgggattttctttgacatagactccagagtctggtataataatcttgtaaacaaaattaattcaaaggagttgttaattatgaataacaaaaaatttcaagaaactttagaacaattaaaggaggaactagaaatacaaggggtagaatttaatgatgagaatgacttaatagctgctgttgaatacatcatagaatatgattaccacccagaacaatatgtggaagatactttatgtaactaccctgaaatgttcaaggatctataaaactaaggaggtgtaaaaacctccttttttatttttctaaaaatctggatttaatcgttgacaggatcgggactatctagtataataatattgtaatcaaaattaattgaaggagatgttaactatggaactaacaagatcagaaaaacttaatgtaataaaaggaattgctcaaaaggctatggataataaaatctatccacaatttagaaaagaactagataaacaggtaaaatcctttggactaagcaacaaagttagggaaagtgaattaggagactacctttcttgctgtatggttgcctatgaagaggttatactaaaaatgaaaaaagccaattaatatgggtggccaaaaggccatctatttttttcgaaaaaatctccagaatctcgttgacatagtctgggccctctggtataataataatattgtaatcaatattaattaattcttaggaggaatgaaaaatgactaaattagaaatgttaaatgagatagaaaaaataaataaggtggtttttgaaaagaacttccaaaaacaattcttggataaggtgatagaactactacaacaaatgggagtaactaaatattatgtatgtaaacatcataaaaaagctgagattgaaaaacatcttgaggcttgcatctgtgcaatatatgatataggaagaagggatgatctaggatggtaaaccccatcctttttcttcgaagtttttcgttgacagatccagagttctctcttataattaaatcataaattaactattggaggtaaacaaaatgagagatatgatagaaaatcaattagctgaatatgaggtaaaggagttatacaatgaggccacaatgatcttaggaaaagcatttggtgtaagtgctgttgatctttatatagaatctgatgtggatgctaactactatggtctatgccatagatcaggtaataaatttactgggattacaattaaccttttccctttcaggtttgcacaggaaggagaaaaagcttatgataaaatcaaaaaatttggctgggatattaaggactgtgttcttgaaactatatgccatgaattggctcacttaacttattggtcacatagtcctttacataaaaaattaactagtctttattacaacaaagtgcaacaggctagaaaaggtgaaaactcagctgtagcacaaactagaagtgatatatacactttaaaagatttatgtgaattaatagaactagatccaagaaaggctagaagtatattaagaaagaataatattgagaaacctggtaaacagtgggagtgggagcaaggtatgcctaaagatatatatgatctattaatcaacttaaaggttaggggaagaaggtaaacttcttctcttttttcgttgacatatctcgagagtgctggtataattatattaacaaataacttagggggtaaatcacatgatagatatatattatagtattcaagtagaagctgaaaacttctttggttgtcaaaaagaagatggaagctgggtagcaacaggagcatttagtatacctgttaatagcataacttttgaagaggctgatcaattatccaatgaggccatagatgggtggttaaaggagtatgaggttactaaggtaataagtaggagatcacatacacaggttaaattagattggtataatagttatatcaaggatgatccattaaagggtgatataattaatatggtgtaccctgatctttcagataaagctaaaatcaaatatggctttggtaagatatgggctagcactatgtcaaaggttgctaagaagggtttacttaaaacttgccctagatgtggaggcactggccattactcaagaacctcagatggtaacactacttgctttaaatgtaagggctttaaatatgtgataccaactaagatctcaaagaaattttataaatctgtggagaaaacctttgacatctctggcaataactcttataataaacttgtaaacaaaaacaaagaggagatgttaaatatgaacttaactgcaatggaaacaaagatattaaatgctatgagaaagaatgaatttgatgatggactagatgttgactgtgtatgggtattctcagtaatagaaaactcaggtatagaaggaactaaggctagaggtgtgatctcatcacttgttaaaaaaggtttagtatttgctgatggagaggtaataggttacacagaagaaggaagaaaggtctttgataatgctgatggagaagaatgtaactggggaggtccaaaattattaaaagaaatccctgacaaaccagaggaaatctcttataatgaaaatgtagataaaacaaataagaaagaagaggtaaatgatatgaaagatttaaatactatgaaagctgttgaaattaaagaattagcaaaggaattaaaagttaaaaactggtggactatgaaaaaggctgatctaatagctgctatccaacaaatccaacaaccacaagaagaaaaagttgaagaggtacaacaaccagctgaacctgaagaaaaggctgaacaaactaaaattactcttgatctaacagatgttaaggaacctgaagaagaaaaggttgaaactaagaaaaaaccaaaaactaaagaaggtgtatttacactaaagatgatacttgaagaattaaatatgaatggtaaaaaggcaagaaggatcttaagaaacaaagaggttgtaaaaccaggaaagcaatgggaatgggataatgaagaagaatttaaaaaggttaaggacctactttctaaataaagtaggcccaacctctatcccctattgatttacaggaggatctgattttctcttatccattaactgcttccatacttgattaccaaaggaagctacagctgcacatattaaaccctgtataaagccattcaaaaaggtcttggctgtaaaacctaattctaattgaattgccatatataagattgataatgatatactgaatatcaaaagtattaatggtatagaccaatctggtatataaggcttagccttgataaacagacctaaacagtaacatgatacaatgattattaaaagctgtggatcaatgtaattgaatattaagtttactaaattttcttccatgataaataccccctaaattatctctacatattttgaacttacataaccttgcttcttaccgtggctagtattatattctatatgataccaaccattcttacttcccaatatagtaactctctcattactaaatactgagcctattatattaccattcacatcatctcttacattaagagaagtgttaactttaactattccttgtttaacatcctcatagaatttctggctttgctcaccctcgtagcgaacgtatccatcagatggagtaccatcctttctataaaatgttattcttaaccagccattagttctatacattgggctagccttttgaccaggctgtagttcttcattatgatctttgatgttaacgtcttcagggttccaccacacataagttactccattgtcattttgatatttcatgtggtagtcaaaacttaatctgctgtaatgttttatgtcaatataagcatggtacttcttattctttccaggatatacaacttctatgaaatttctagaaggatatattccgagaacaaataaattatctaggctatcaataaatctaccagggactggcttacaatcctcatctagaacttctattgaaccttcccccactaaagtagcattagttcttgtctcattagactcatagaatcctttggggttattgattactggtgagcttgagctctctcctgaatttactctttctaggaatgtattccagtaaccattggctatcattcttctaggacaattttttctactggcatcatagtgtcttactactttacaattagaatagtagccattctttaggtatctaactagctctacagcattatcaactgccttattgtagtcagagtcaggattaacacatatttctatagatattgtatttctattattgataccgtatctattatgaccatctccacaattccaagtggcgtgtttgtgttctacagcttgatatacccctgtatcatcgacataataatggacactggctttacctatatttccatttgcttgagccttacagtgggtttcggctccagcaccccaagaggtattatcagtttcgtggataattatatacccaggattatttgcatttagagtaacattcgtagtacttaatcttttattgattttcataataaacatctcctttatatattatagtgttttattgggcctgagaggctcgctacagcattttaaccacctccttaatatatttccttatataaaacctaacaggccttaaatggcctgctaggcttataagttaacctttgttactaaataggtgatcttttatagtatctacatcctctttgatatcctcaactacattgaatttatcaactagcttatctatcacttgatttaatttattctccctttctctagcttcttgtctagtgtcatataatagccatacaaatagactacaaaagataccttggctaagaacttgagttagtatttctttttccatagattacaccctttccttaaagtcttcaccacatattcttttatagtcctctggtgtaatttctccttccggattagaagagcattttaccgcctgatgtaatttgtccttacctattgctccaattctataagccatttcccagaaattcataatccctacctccttatttattcatcattttaatctttatatcagctagttcttgtgttaatactttcattatggccttagtttgcattagctctaatttagtatcagcaagagcctgggcttgataaccaattaatttattaatatccagaggattaggatctatagcctcataggaagtaaataggtccttatctttgatactgtatagatctgatctctttttactaatatcaaatttggttgggccaccctttatgtggtcaaataaacttacagtcatttgtatggctgaaagattgtctagatcaattacctcagtgttatccacaaaggctaaatgcccttgtgaattatgaggtatatggagacatataatatcttctatattatttaatatttcactatcctctctatagtatagaggttcaggcctattaattaggtctaatatcttagtaacttcttcatggtctttatctataaatgattttacatcttctgagtcttctgcctgatttatcagcatttctttttcatcatcatagaatataaggtctatgattttattagtttccacagaataattaaatcctactattctcatgttttatcaactcctttactcagtggctaaataggttagtattatttgagttggcttaccagctaccatttgataacatccaccattcaaatatgagttattccaatagtcaatagtacaataacctgaggtattattagaagcgtcattatagttatgtgatactagagatataggtaatacccaattccaagccttaggaaaatgtatagtataacttacacctccacctgagttagcataacccgtcttaactatttgacggactaatcttagtcctcccccaagatgacatactctaacgttaccattgtcattatcccaataatctcctttagcaatagatctattatttacaacgaagtcagtaacattctcagtatatagctttttgttctcttgtttgaaatacaatcttccatcttcagctccaccataccagtcatttattcttaggtattttctagcccataggttttcagctgatagagccttatcaacctctagagatccgtctctagtagttatcctcatatcaaaatctttcttactaccctttaagtggaaatctaatataggacctagttccataactccatcatgtgatataaaagggatacctgcatagtcattactagctccagctaagtcccattcttttagtttattactgttagcagctgtagcggttttacctaaataagcactatcatggttatggtctgaggctgcagctcctatatcggatggcttaggtttattgaggttactataagctatacaccattcggaccatatgcctttaaaactacaaaacctagtatatgttttgccataactatctgtaaatagttgagttacctcaccccccttgggtaataccaatagagttccataaataccatatgtgtaaactacaggggagtttggtaaggtatctacactagatactgagtatatcccctcttccttacaaagattaaaatctactatatcatcttttctaatagttaaataaactccctcatgggtatggttagttggggatgcccccacatctgctgcagttggtttattatcttcatgatagaccttcttattgttcttattaacaatatccagagagtctatctttacaggccttccagcataccctatatggactttattatctgcatctatatagatcacatagtcatcactgccttctttagtcctacagctaaatccataattgtgggccccaataaatttctgacccggtctcatgattagatggcctgataattctccacccgtagtaggtaaggcaccaatatctgctggagtaggcttattttgtttactatatatttcagcccaattcgtccatccggtaccctcaatgtttgtagctgttctagtaaaaactcttccaccatctgcaaagaacatttgagaagcccagtgtcctgtattccaggataaaacaatcaatctcccatctgctaggattggggcatttctatcgacagaatttctaactgtagaataaatacctccctctgtaatggtgtttagatctacaccctctagtcttttggctgttttatcccaggccccaatatctgcgggtgttggcttagctccggagttataatcttttctccaagggaaccaatccgtattatttactttatacctccaatacttattaccattagtatcataatactcttgccatatccagttattagtattattatgcttagtctctgtactaacatatactatcagtataccatattttgtaccagttagtggggcattaggtaactcacctgagatcaggtattgcccctcagttaaagctgtattaaaatcagttatggcgtccttaggaatgggataagcctttaggtcagcaggggtaggcttattagcctcatcataaaccttataccacttactccaagaattatttcctgatgtgtagtttctaacatatctagttattttattggttgggtataggttaataaactcctgttggaatcccctctcacctgtatttctaaccataaaaaccctattactcatatgggctaaggttccctcgggggtatttttaaagtcaccagttcctgtatcaaagtagaagaaggcattcgcttgtttaaaggaattacaatctctatctaagggagcactaaccttaataagtgcttgatcttgattagcctttcggtctacttgattttgtaaactggtgtctttctcaaataataggtctaatctttttagcacatcctcaggggctagattataatcaggtactacattacccctagctaatatgaggtttagtacctttaatgaggtacttgaggttgcactctgtaccacaaattgtattttggtatcagtagctccagatggaatactaaatttatgagtttttaacttgtacccattactctgtggtgtactaccttgttttacaatactcctatattgttgacctccattagtgtaagccagtttaatttcatagctagtaaaactaccttcaatatcttctagaaaggctagtatataatcactatttggttctataggcagagttttaatctcaagagtttgtggacctgttgacataccagaccatttaaaacctcgtctctgggttggagtatctgtaatgggtgtgatattaccaggaccagtataagactcagagttgtaccactcaagcctattaatagtaccaacccttaaagcatctagcctatcctcattagacttagacttcttttctacctcagtcattttctgtttatgttcggtagcaaagttctcaatgttctcattgtccttgttaaaatcattcatttttggcttatctgttaactcccacttatttaaacctagggtaggagttttactagtacttggcattttgcatacctcctttattcagttatagcatattcttcccatttttcccaggtaagatctagactgtcccacttgctccacatataatcatatctatcgaacatctcccaagtaatataaagtaatataatttgatatattaggtgagcaggcattcttcccctgaatactctttctagagcctttaggttaggtggtacccctggtaggtcagtaaagctaatcttgatcttactctcttcagctatgaactctacctttacctttccacctgtataggccttagtaagatttttgatagatgtactattaaactttttccaagcagatagaactactgtaataatagctcttttctcttggtcagttggtgggtaatcaaagtatttatataactcaagatcagtaaaaaatctttctagaccttccttaggagtggtcttgggatccacatagtcttgtaattcctgtcccttagtatataacttctgaagttcagtagccataatggtgtttactaagttatcagcctcttttatattatcataaaattcaggaacatacaatagtaattctttttgaacctgttctagactatacataagttaccaccacctcagtaatggttggtatttgattagcaggaatagttaaagattgactacttccattaagtgtaatggttgtataatcttctactccctcaatatttaaaagcatagcccctattctatttatagataggctagtaattttaaatacttgactatttagaaattcttctagttctttcttgaagtttaattttatttgttcttctgtaactgaactcaatttcttaacttgagctcttacagtgatattaaaggtttgggctgactcaacagtaaaaacacatcctataggagctttaccctcacctaaacctttcttgcctggatccatgtattcttgaactttattaactagctcaggattagcaggcttattttcaactgtggttataatacctttagcagtatttattccatcccaacagggaagaaccacagctttacccactccagctacacttttacaccaatcagttaactgttgaacattcccatctccagatggttgtatagtggctttagtagctctttctcttaactcatcatctgtctcctgatctctaccaataacaagtatatctcccatagtagcacttctaagttctgctatagcattgataggaattaaatgtgtacctgttgatactttattgggtcctgaacctaaggtctcacattcaataatattaggctctatcacttgccagaaataatctcctccttggaatcttgaaccaacatcgggttcatagccaacaaatatagctgaccttctacacttagttggaattattctggatatccctacattggcagctctctcatctaagaacttacctgtagcagtacttagaaatactgagtctaatatttgattaacattaacagcataaaactcagctagcttaacagcaaaaaccatagccatatcataggtgaagcttccagttctagtgtcaatatcatcaggggataggcctatcatttcttctaataattctttatgtgttcgggagaataaatcttcagaaaatcccattatatcaccccttccagttttgtatctccatatatggtatttatccatacttcaatatatacattcttaccttgcacattatactttagatcagttactttagtcactctatcatcttctaagagacattcagggatagccctattaatctccatttcaagaagttcaggagttactagagagtcattaatcaaagctctaatatcacaaccataagaagtatcttgataaatcatataggcatttttaggagttattaatcttttatataaagattgttttaaggcctcaagaccatccacattatcataaatcctattaaggtttagatccagtttataggtcttggtattctccattgttttctcatcaactataagagtatctttaaagccattaggtagcattatatcaacctcctaagatccctaacataaaatatctttgtccatcatcatagggcataagataaacagtatcgccctcactaatagactcaatatgttttggaacatctataatatttccagatagtactaattttctattgtgaagacactcacattttagagggctagtactaagtaccttagctctataaatatttagaggggtggacatattactatatacttgttttacacagtctaataaattattagccattaaatatcaccctcctcagtacatttaagttttaaattcatggtgtagtcagtatcaaatttatgggtatcagactcaatgtagaaagccttgttaatttttaaatgtggtatactaaccacaatggctttgccactaatacaatcaggtacacctataacagttatagagatatcagttttaggtctcttacctgtttctagctttattctagccttctcatttaattgggcttggtttagttcatcactgatagtatcgtataattgaaatacaccatatttcttttggctgctatcatctttagcagaggcaaataaagtaatctcgggatcatctttacccttaccctgtttatatttacatactagctttacctggttgacaatactatcaaagtttctacttcttgaaaaggttccaatatttttaccatattcgaatttccacaattcattattggttcttcggtttataaaatcaaacttacctgtaatagaattatagtaaatataaaactgttctccagtttgttcataaacctcttttattaccttcttcataatatcatagggagtttgtttctcacatactaaactagagaaagtatatccagttttagctactactccaggggcaaccccaaaggctttacataatgactcaaatatagcttcgccagtttggttttcgaatacaaagctatctttattattagcccaataaatcatagggtcataagctttaaccttaagtaaatgctttttctcattatctgagatattcataataataccattaaagatattcttaccctcatggactagtactacctgatctccatcataaattggatgtatatcttgagcattatattggaatgatagggtacgaggggcagatgaagaagaccctgcccaactcttaccactggaggtatttgtaatatcaaaggatttatctccttgtaccacaattaattgcatattataacctccttatataatcaccagaactccaaccttctttatatcctgaaccattatctaatttatactttacataatgccatccattttgagatcttaatactgtaaagtgttcattaggccatatcttacccttagtgggattattgatacctggtccagttcttacccatagccatgagtaaacattagtagtagtagctgcccaaggttgagtacctccagaagaactacctcctgtattaccactataggctagtttaggttttggaattgtaaaactaactgatttaacctcaggcttcttatactcagttagttttatttttacttgaagagtaccaatatctccacctttctcagtatatgagatattatcaatagtaactaataagttaatatcagtactagtaatagtaaatcttactggatctttacccatttcaataagtttagcataacttactctagggtctgcaatatcagtatactcacatccatcgtagtatgagcttggtaactcaaaattaaaagaaaaagattttagcttagggtctcctatgaaagagagttcccctaagccttcaatggaaactgtactattatctctactatcagagatatttatatcagtgggatttactggtaacctaaacctagtatctccctgtattaaccagaattgatatttactatgcaaggtccagttcacctccctcgaacatttcctgatttaacatttccacaataaatctgtatactctcattaattcactttctgagattgttccatcttcagcctgtactgtgaaattaaatgagttgttaatgttcataactttagatccatcatcacttcctgctccagattgtcttagtaaatcctgagttttatctgcaggtaatacttgagagcctctaggcatttttgagaatgtaggacccataactaattcaggaccagcttcaccaaccatggcagctttatctgtaaagaagtcagtaccttcagcaagcattggtatctggggaatattaatacccttacccccaataataggtacccagtcaggtatcttaatagtattaagagcaccaattaagttattaatcataccaataatactattaataggagcttttgctagggataacataccttggaaaatacccccaaagatgttcttaacaccttcccaagctttagaccaattacctgtgaatactccagccacaaaagctattaaaccactcaacatctgcattaatccctgtagtattcctgatatagtttgaacggccccagtaacaactgaggagataacaggccatactgtttggaaagatgcggctaaaaggttaagtagtggagttagcatatccaccaacccttggaatatcataccaaaactctcaatagctgattgaatatatggaactacattctcagcaaagcttaagaacataggtagtagtgtattattccaccaatctgctagtccttgtaatattggcattaggaagttacctatagcttccacaacttgtgatatagctggggctatgtaggtgttaaaggcttcagctaatgatacagctattggcatgaaaacattagttatcaattctccaagagctgtaaaagtagcagagaacatagaacctaatacttctaatatagggcctaacacttccaatacagtttgccatacttgagtaaagccttgaacataaagaactactaagtctatggctggaattaggttattcataaatatagaagctaaagttccaaacatatcaagaagtacttgacctataggagctaatactcccatgataggctcagctaaaccattaaaggcttcttgtatattattattagcctctgataaataatctggtagacctattaagatctctccaaaattattatagatgtcttctccaagactccatatcttctcattaatttgatctgccacatcagcaggtaagaacttatataatatatcattggttagatctataaagggttgcatagcatccccaaactcccaaccattcatgatgtaatatatagtctctcctaaaccttggaaagcagaaacaaccattgagaatataggtcctagtttttcaaagccttcttgtataaatgtgataccatttagaacagcattagctataacctcaacggcaggggctagggcatctcccacatctaacataactacagcagctttggtttttattctctccatggttctattaaagcccttatccattttttcataggcagcttcagtggccccagcactatccttcatctcattaagagcattagtaaaggcctcagtaccttcaccagtcaaggctagtgcagctgaaccagcttctacagaaccaaagaggtcattgatacccagattacttttctgggcatgtttttctaacatctgaagggcctcttggatattacctccacctttaatgaagtctttgaagcccttaccagctatttcccggaagactttatcagtcttggttcccgatttagatagctcatctatagcagctcttatcttagtagtagctacagatgttggaaccccctgagctgttaatgcagctatagaggcagatacttcttcaaaagataccccagcagctgaggctgaaggtagcacattgaatagggattgtgatagttgctcaaagttagtcttaccaagtcttactgtagtaaacataaggtctgaggccctttgaacatccatattcttagctccatatgagttaataacagtagttagtccatcaaccgcagtttctattgatgtgataccacctatagaagctttaccagctgtttctaagaaactaaaaacgttatcctctggaactgatgaggatatagcttgataaagagcaggtactactttatcaggcaatatccctatatcagaacttaacttttttacctggccggacatcttatcaaaggtctcttgagtagagttgggtaatagagtcataacctcatttaaaccttgctcaaaatccccaaaggctttaacactgtccttagtaaaatcccagacagccttagctgagaatactccagcagctactccaccaattttggcaagagtacccatgaaggaattaccactatcagccatctggttaaatgcaccagagatcttatcttgggcagagaatatggcagtaaatgccgcttgacttgccattatatccctcctttatgattaagagcctttctttaacttatccctagcttttttatcttcctctaaagccagttcacatgaggctataagaaaggctttcctattgggagatagtttatcaaattcccagggtagtatattatgcttctggaataacacatgagcccaaaatgcactagtgtcggcctttattagttttttgcttctttgattagatcatccttattatcgcctaatccatttatgtccataacctcactagttattctagtgaaatctcctggtaagcttagtacatccataagtaaatctactggatccacaaacttagtagactctaaccattttggatctttaaagtcagggaatactattgtttctagtatcatttccctagtagctcttctttggtctgttattgagttagttatacctttgtttctagtaattactgtatttctcttttggatatcttccatttgcttagtagtgattggctttaatatccaaggtataggttggcccgctaattcatgaccctcagggaaactaaatctagctaccccttcaacttcaatttcgggtgattgtttacccttatcattttccatgaaaaattccatactaaattttgacataataatctacctccacaatattcttaatcttttataaatatcttacttctgaagctgagaatgatatttcttcttgaatttcttctccctcagcatctagtccaattagtggtaaatctccttctaattgtactcctagtaattgtactctgtcctcaccataattcttaacatagtcagaatctggatcatcacatacagcttgtatatccatcttagggaatataccagtttttaagtattccttaatagcttctcttatcattggagtagctttgaattgagttatagttccagttatatcataacctataacttttgaggttaatcctttctgacccataactcttttcttagtcacctcaggagtaaatagagcttctagttttattaagctagttacttgcttacctgatacaaaagctctaccctctctagcagacattctattaacttcactcatgggctatacctccttaattattcttaacagttacaaagtatttcttgaaagttcttacaggttgtgtaagtatagtagcatacatagtctttcctttactagcttcttcatctaccactacatcagagtcagggtccacattctttaatgctccttgagcttgtagtgtagttaatagacttattagtctatcctgagctagctttataccatctttgtggttagggaaaacattaggaactaagatctgagatcctagatctataacagcatccaatacagccacaactttgttatctgtaaagctttcatcccattcttctgtaaaagtatggtgtgtatttatatcttcctcaactactacctttactctttcagaatttgagtcagtttgagttgagaatataaattgacctgtttttaatccatcaactatttgagagtgttttagtcttggattggcatctactgctccaggatatgctttataagtaaggtcttcagtatatccagctgcagctctagcaccagctacccatgcagttgcttgagaagctgttaacttagtgcccccttctaatacaacaccattcttaacattgataatgtatgggtaatcacaagtagcaaagtcagaagtaactgccacaatattcttaccaacttcatctctgaagtatttaagttttgataatagagcagtgtgtaattcactatcagtaaatgggaaggccatagttttaaagttgtataactcacagttatctaagaagttgataacatcagagttattcatctgagtagaagtaccagtactaaactcagtcttagcagtctcatctatagaaccacttccacttactgtaaaccattgagacttaactgttgatatttcagttactcctgtagcctcaaagattttagatccctcaagatataataatatatcctttcctccaagaggattggtcttaatagttagagataacttattacccctttctccagctttagtagctgtaaatgttagagaccctactacagctttggctttagttccacctgttaggttatatactaaaacagttgcagcttcttttaaagcctctttaactagtaatacagtagggtgagttatgtcatacccaagttgatataatgcttctaggccaccttcattggttaccttgataacatctccagcattaccccatttaagttgtaatggtaagatcataactcctagattattaagcttaggctcattaagtccaccacttacgaatctagtatacataccaggtcttactttattttgtcctggaataaaagttcctcctgccatctattttacctccttctttagccagtcttttataatctgactagtttgttttattgttaactcttcatcaggtggaagggattgaactgcagcgttgaagacaaactcctcaacctggaaaagttgttgacaatgggctcttaattgaggtatggaaaatttttgtactttcactattttaccccctttgttatctcaaagttttcgaagtaagttggatctttataaagactaaccacaatatcatagtttatctctacctgagaatcttcttcagtttcaccttcaaatacttccacattctttattttgagatttttgttggtcttactaccatccctattaagtataggaatttttctatttctcaagtatatagcattagctatattctgagcaatttcaagagagtctttaggttcaaataccttaactcttaaagtattctcagttctataactacaaagagtatcattctgaggattaaataccttcttgaaatataatgagggatacttgaacttttcaggtattcgctcaaaatagaggatagtaattccagttagatcagatatgaatttagcaatactccctatatctgctgtcattaataactaccccctaaaacttcggctaaccaatcttctaattttctttggaaagcctgttcaaatattttttcatatatttttactgcattgtcccaataaggtttaccaggtactttcttttgtcttagtaccataccagtcttagctcctggttgataaataaatttatctcctgaccatatgccaggaacgaatctaaatgattgtccttgtggattagtgtagtgaccatcgtttacccacttagcatattttaggttagtaccaacttctaaagttagtcctccatcactacttacccatataccattcttacctcccttttgaaaggagttaagtaataatctagtgtctactacttgtagtctaattatttcatcttgaaccacatcaaggaagtctatccctgcagcttcaaaccatactgctaattgctttttgaaatcactattagctgcatctcttagcttctttataaacctttctatttgtttagcatctatttctatgcctccagaatttgaagccataactatctaaaatccttagcctctataccaaccttaatttttagacctcttatatccctaggagctttagctatatatgtgataccagtctcaaggtccacaattttatcattttgtctaacatcagttccaatagcaaaatctactgagtactcctgggtaatcttaaacctaggttctttgtactcaagtttttctagagttcctgacttaaaatgacagggtacctcagtcatgtctggctcatcaggataactaaagctaggggtatgggctagcccatatccgggatcttcagggtcttctaataggtggtatatattacatctatgatttaagagcttgttatatgaatttccaatcatattacagtacccttaatctcatagtagttgttctgatagatggactatcatcttctaagaaaggtttaatcagaggcataatatcaggctctatgacagccttatcagttcttcttgtatatgagtaatcatcataggtctcggattgaatatcagccttgctaatgaccaaggattgtagtccataatactcagcatacaatatatgggctaaccttaattctttactattaggatttttctccacaatagtatcatagtctttatttgaatttttaaaaattcctgagatcttggctttagctcttagtatatccatctcaatatttttggggtctcttttcttaatctcaggattacttgaaaagtcaattatttcatccggagtaatattcatatgagccacccctatctgtttcttttattcttgtttgtaaatcttctagcaggttcttctttactgtcatctgtagaaggtatttcttctccagtaaaatcttctagaggttcatcctcaacaggttcatctatgacaatcacatcatagttctgttttaaataatttactaggttatctttaacttcttctacatggtcttgagtaattctatgacccttaataaccagagtttgtaatttaccctttgctaatttgaccttagccataatatctctcctttctaatgaaaaagagcccacatttatagtgggccttcatgattaagcttttaccttgattatcttagcagcagctttaggatcttcaaacttaacatccatcttaagagttaaaactacataagtagctctttctctaggagctctttctaattcaattctgatatctcttgatatacctataactatattcttagggtgagttaagattatatctgatacttgagtagaagtatcttcataatcttgtagcatagctatacctttaacaggtacaccataagcagatttaacagagccatttataaatgagtcatcaccattagcagttaatctctctcctactaagtctacccaatcagtttctaaaccatttgagcagtagaatctccactcactggggtttcttaaatacttagctggtacagctttcttagcttgttttaataggtctttacttaaagcacccctttgagcatctactacatgagcagttaactgttttctaaccccatctaattgttgtaagaactcatcactaccctcactagtatcaccattaacaattatttcttccatatcaagagcaactctttcagctaataattgcattacagtgtcttctattgattttccttctatatttgtttctatagtatcatcagttaacttaaccacagctataaattctttagcttgtaaagtaactgttccagtagttggagctgaatatttagactcccctggatcttttccttcagttgcaggatttaatactctttgaccaaatcctattgactcaatctttttagagtctcctttcattggtacagttctagcctcttttaatattgttggctcatcaattatcattttaataaaagcgttagcttgttctgtgtttaatttacctccaccacttaatactgtagagttaaatactgctttatttattttagccataatcttttcctcctatcaattattcttggtttccaccaaataatccattaaatactgatttttgaacttcttgtccttctcctccatttttaacaatttgtttacttcctacatatggagccatggccttagctactgcctcagctattttttcttcctcagttttttcttcttgtttctggattaagccagcctctaacatagctttttccacagccttagcaactatatcttcagtagtagcttgttgaccttcactctttttaacttcaccctcaacaggtttagttccatctaatgcctttttgatagcttcgtctatcattttttgtacttgagtttcattcatctcttcttccccctccactgagtctaataattcattaatagcactttgtgctgtttttaacttttccacattttttgaagatattttcttacctgccttattgactggtaactcaaaggatttagctacttcctcgggagttcctaataatattccctccatagtttcagaaaattcttgaagagcttcctttatcttatctacatcactttcaaaagatctagtgtaatcccaactagaatatggatatagaatatcttctaaggtactaactgcattccagaaattatccctttttgcagtctctttatatttttcagagtatgcacctttctgtatatgctttggagttaaccctaaggcctttccaatcttatcaagtatagattgacctatagacttctcaatctcatcaatatctacatcttgtgtagaatatttaccagtaccacccatagaccatccagtaatttcgcctttctcaatcttgctccatagatcatcatcgacaatctcagctttagctagccaagttccagctttaactactgtaccttctattgtagtatcttcctcagttacccatgattttacaatcttgacaccctcaagagtgttctcattgtgttgtaaatcactaccaaggccattttcattaaaccactcacaagctttcttgatctcttcctcagtcataaaattatcatggtagtcagcagtcattggctcatatactacaccgataacaaaatgattatctccttcagactcagactttaagattggcttatcatatctaaatctattaggagccccaagttctttagccacaatccattgccatttattagctgctttatcaactaatgaaaggtaatcaattttagcatctgagatctcaatagctttcttaactgattttactggcatttactctccctcctttacaaattatattctgctatcacttgatctctgatagcttctttttcttctttagataatcctagtatatccttatcaattacaggcccatgggtacaatgacaattcacagtctcagaagctggtaagttgatatccctaggaaatctagcttcataaattcctacagtgaagtactcacctttattaatgacagtaccatccagatcgacatggtgttgccttgggtgaataccccttccccctgagtgtttccactgtattcctgttactgcggggcattgattaaaagcctcatccttagcatatgaatgagctcttaacatttcagtaatagcagtagctctagctctagttctactaaagccataagtctcagataatttaccaactacatcttctacagactctccatcttcaagagccttatccagaatattctgtagtttttcatgggaagttaatttcatcatttcccctagtttagaagaccactcatctataaaggtagtagtatatggagaaaagactttggttagggataagtccttatcaataccttgtaaataagtatctcctaaattttctatagcttcttgataacaactcttaagagtttctgctaaagaagtatcgatattatctgtacctatttgagactccacatattccataaattcttcaatggtttcaaagtctccatcttttataagatgttttaattcttctgtaaggagatcagaaatagtgtcttctaattcagagatcttttctattgtataatcaatctcctcatagccagcttctttcaattctttcttaaggctatcatcttcattctttaagatcttatcaattttagcgatcaactcatcagtacccactattacttacctccttttaattgatagtttaataactgtttcttagcctctttaagtacagctatcacctcatcactcccattagagctttgagccttctcaattatacttgttaagttattactcattgaagaggcaactgagtaagtagggatatttgcccattcttcatcaataggagtatagtccttattgattgatgaatagtactcctcattaatctgattaggagtcatagctctagaggctatagcaaacattcctttctgataatcagagttctcaatattaggactcttaaagtaagcttccacatatttaaaaccatagccagatagaataacattatttagtatccatgttaggttttctctttcaggaacaaatacttgctcttcagtttttcttgtagcctctctggctgtagccacattataatcttgggagtaccctacatatatatctggtagtaagaaagaagattgtatctttttcctagtattatccatgtagtcttggaataactcatccttctgtaatatttcagataggggcttgacctcaacagtaactggcttagaatcatcaagggcagtgtctctctctgcagcttcagtttctaatactaagaaaccatgctgggaattttcaccttttacattattcatgtactcagttaattcattccaagatttatcattaagagtaccaccttgaattagtaacattaatggagtatgtttaccattagtaaaatatctccagtttaataattcggcctttcttgaaccttgagcggctaacataggaccttcccatcttggtgtaccatagacaccataacctgttttaaaatgaagtatactgttagctcgatctttaagaggtatctctcccttttcataatactttccagtattcatatctagatctctaggatctccccactctttaaagaagattgattgattatttacagtctgcttaaatcttctgaatctttttcttctagtgtactgtttaccatatcgggttacagtgtactctgtactctcatcatctagcttaagaattttaattgtcttagggtcttcaatttcttttatctcttttacgagagctgagtctttaggatcttctacgatctctaaaaaagaatacccaagtccttctctccaatcaactatctcttcaaagacattcttggttggtttatcaaaagacagggtatcaattaattcttccagctgtttatattcagcttccatttctggagtaggttcatctaccttctcaatatacctaatacctattccgaatccagcaatattatttcggtaggcctttttgcattggggtattattgtagactcccttataatcacttctaatagttgggggtcatattcaggggatatctcatcaacttcaattccaagtacactggtttgttgattagatttatccactggatccaaagacttttggatagggtctccacatatacttctggcggatatctttttcaaagttactttacctcctttcttaccttatatatcaaattataaaatccagatggcctcatatttcagggaggattacatcaactccacatatagtgtcaaatacggccattcacatgatttaaaaataactataatttgatacgtttattataacataattcacaaaaatttgtcaacgttttatttttacattattttccagaagattttccgcatatattccccatataaaattatataattattaatgtatactatattactatattaatttatgaaataaattatatagtatatagtatacttatattacatatatataaaggtggtaactctgatatgccttctatatcacattattactaatatagagcctagtcaatttcaaaactgatatctcacatatcagaataaaaattattggctttaataggcatatcagttacttagatttttcttaatttagatccaacaggaaggcaagctaagaatagagagtctgctaagtctggagaatgtagtcctcttttcttcatttcatccttactctccagctttatttgacctttggagttgaatactttaaactttctggtagtcaattctcccacaagatctgtattatctggtagtcttaactcatcatcctccagtaattccttaactacagaggctatatatgtggttgtatcataataaaaggcataagcctgggaccccctctttaatggcataccaaatttacatggtactaccttcaaccagtccagtttttcttcaaattttatctcctttaatctatcagttactcccccacctacaccagtgtcgtctattttcacaactactgctagtttagggaactcaccatgtagggatttagcctttcttagcacttctcctactgttttcatagtgtccttaccttggtaatagataggttcttccacatatccatcaattttggtcataatagaggtcttatctgaaccaaatctagctacgtctacacccatatctatagtaactggttctgtaggtctggttatttcactattaatacctctatatactgtggataattgtataaatatgtcatcttcttctagtgggaagtccccttttaccagacatctgtagacattggactcttctccatactttttccttaacattttatggttttctttatcagttctatcaacttttgtagcgtcaatatgaatacatttaaaattttccttaagactgtggtgagaatcaaagaagatacctgtatttttaacagggttaccaatcaaaattatcttattttcctcatcggatatagtaccaagtaatgcttctagtatctcatcatctattccaggagcctcatcacatataattagcataaactcactatgaagaccaagcatattctcttttctattactagttttacacatagcaaaccaagtcataggactacaattcctagtcatagtagttttatttactgtaaagtaatcttccacaatagttccttgtagccattttgatatttcaggccataatacagatgttaactgtgaaaatgtaggagctgtagcaattaccttacattcaggcctaaaggtcatataccaaattataagacaagcacaggccatggtcttacctaccccctgtcctgaccttacagaggttctcttattgtctcttacactcaataaaatatctttctgatgtggatctaagtgtactcctagtatatcttccgagaatccacaaggatcgtcatagtatagatctactaattcttcaaaggatatttcttccagagcttccttgttaatgtggaacttatcaactaaagcatctagctctaatttctcaattatgctatctaaatcaaacaattatatacacctccttagtaaagtgctttatttagtcctgtaatacctttttacttagtggtattagattttcctttacctgcattctttttctttctatcagccattttggctctaagaacctcaagatcttttcccttaccagcattattctgattttcctgtatttgtaaaagtaatttaaccttttcaagttcaactttcatcacatcagtacttaggccgaagtatacctcaagtctttttagtgcctgaagtctatcctccattttaactgatacgccatctttactttgtttaatctcattgattaaagtaccatctacagccttactagaccttaatagaactagatcatccttgaattggcacacatcagttatatctgcaaaggctattttcatgtactgccttattacatccataccatcgcatagtaattcttcatctctatcggctctgatagcctttagagcttcctgtattttcttcttctttaatagtttagacccatgtgcatgagaattattcccaggataacctgctctagcagctgctgtagttgcattaaagcacttcatgtaatgaaatacaaacaactcttctttctcatcaagatcatacttatcagccagggtcttaatagtcttttttgttttgctactcaatgccacaatatcaccttcttcttctaaaaatgttatgccctgctctttaaactctcttagacactgcctaacaaaggtctgtgataccttagcaaggtttcttagttgtttaggatgtgtaaagggatcagccttcagggcattatatatcaattttttggctttcttcaaatgttcaggagtacagtactctggttcagtgtatgacttatagctcataatacaatatcacccccttaaaatccagactttactacgtgaaaaatggttggcacactaaccttaatgctagtaataccaaccaaatggcaaaattaactatggatttataccactattataccacatctggattaattatgtcaacgttttataattttatttcacctgtcaatattttttcatacatatccacatctattcttccttcctgtagcaggttatcagctgcaatttgtatctcttctggggaatatactggattacctttagtatcaagttctataccagtatatgagtctaccttacctctgttcataccatatccaactgatttatgaacttctagtttttcattatggtcttcttgccagtgttttaattcttcctgatattccttattctcctctttagtttgtttacattcaataggtctattatctttcatcttttgctttagagctgctgtattgggtttacagttcttagatcctccacctgaacctctattcttatcttcctcataagctttattaatctcaatcccaattattagatccatcttctctaccaagtaaagacattcttttactattggattgttaggttgatttttagaaatgatgtcttgacactctttctttaattgatgtggattattacattggctagggcatttttctcctggcccatatggaattgtatatgctaagcagttacctgctggatcccttctataacatcttcttttacatactattttactcatggttaatacctcctaatatattttctttctcttctaataatttttcaagttcctcaagattttcttctttatcactattaccagctttagctatatttagaatagcttctagttgttcctcactcaaaaactcctttaatttctcatcctctaatatattagatacctctttactcatattgttctacctccacatcattacaaattaatttagctattccctcacttaatctgtatttctcaagatataccactttcttaattcctgcattgattattaaattagcacagctctcacatggggataaggttacatacatagtagttccttcagttgagatcccatgtttagcacagtaacttattaagccagcttctgcatggatcacaatatcacatccaggacctaaacaagttttacaatgttctactcctgaaggtactccattatatgaagtagcaactatcctgttatctctaactaatacacaaccaactgcttttcttaggcaagtagatcttcctgtcataagtttagcaacttccatgtaaagtgtttctctgcttattctgttgttattattttccatagtttatcacctcaattttattatatactattccctatcatatgtcaagagaaactttagaaaggtatatcaccataatccagatcaatacattgggctggctttggttttacttttttaggctctggagttttcttgactttatgatactttggagctctggctaaatccttttttaactttctgactctcttcatatcccactcatgtatttcatggtctctaaaatattcattcaatactcttactgcggatctctttgaaggtgtctttacagagcagttattaggagcaagacagcatcctgtctccttatctgatatagtataacatactgtattatgaggggctcctacaggcctatgaatgaataaggttctgcccatataatcaaactcacataatacttccacatatcttttatactgttgtccctggtcattcttacataatacataagtatattctttcatgttaattctcctttctatgttaaaagggagatcatctctccccttaatatctttttattcttctgttgttctcatcaacctcaatcacttcataccttctaaccttatcagatataccttcctcctgtaatactttaggaatatatcctatggcctgtcttttgttatcaacttcaaaatatctggtcaagatcctttttgatgttacaatcactaatcttactttcatattatctacctccatgtggcctgaactacagctccaggtctatgcttagcttcaatcttagcttcttcctcagtatcaaaatagattatatcttccttgtgttcatccttaacagatacccagtgtactcctaaatatttgttatgtgctaatacactaacatcagggttccaatccacatcaactgtaacttgtaaaacgatatatctccttttcatatcagttctcctttttgtatttatttgttgattttattataagagagcctcggaagtttgtcaaagattttctcgaaggaattcgtataatatcttccgagctgagcataatatagactataaaacaaaatcaaggagttgtaataaatgaaagataataatttaataccattaagagatattgccaaagaggttggaataaatgaaaggaaagccagaaagctattaagatcacatgagaataaagcaaatcacaattattattggatgtttacaccaagagagaaaagacatattgtatcagttctaaagagactgcaataggttttctaaaaataagggagggattaaccctcctttttataattttttgagttctggaaaaatccttaattagttcaagtttcgtaaagttctcttgatcttttccattctcttcttaacttggatagcttcttcttcgcaaggagcatggccccctaggaattggtgccatcttctttcaagttctctgtattcagattgaagttccatgaactcaagtgaatgattgtccatactatcacctcctcaacactattataagtgatactgtcatattctgtcaaataaaaaagagagaatgttattctccccatcttaatatctttatagttgctccatcaactcccttgccatccacatcatggacatacttatcaagtctcattgttgagtcctgtataattcttttgtcttctctgtcaaaaaccttaatgacatcagggttacccctgtcaatgatgtaagcaatctcttgagttccatctgcatatgttacttgaagtaatgaatgtagaggaataaagtctggagctgcccaatcaccaatcttaagatcccctcctatactattcttggtctcatatcctgccacatctgtaggctcatctgatgagtaataagtaacttcaactttgaactccattcctttaaatgaatttatcatctcaattagattttgtttatcagttctcagtttatcattctgatattttaatccttctacattgtccatcagtatttcagtctgctcagttaattgtttattcgactcaatatattcttggacagcatttccccaatgattgtttaggctctgtatggttaacagtagccctcctatcacaattattgttagtaatgacataattcttttaatcattctcttttaactcctttatttttaatttgaatttctcaattccagatttatacttacccacaatatcaaaggtatcggttagtattgcataggtttccccatcagaattaaatctgaagcttcctctcttgatgtctcctagcttattaaaggtcttaccctccttgtccagatatcctttatagtccatatagcacagacaagcagtaacaaactcctgcttattcctgaaattatgcttgatacccataccatctacccatttacttaatacaaatagactttcattagtcttctttactttactattctggattagatccttccacacataatcattagcctctttaaatgacttaaatctcttgcctttcagtatcttactactctggatcttggctttataatcctcaaatatacttggccagaagtcttttagatataaatacaaggaaatatcatctaatttagcattcggatcgttaatctggattacaggatgaccatccattgctctgatattattccttagttgggtattctctctcttcattttagatacttcaatatataatttaacgaatgcgtcagacaattcatgattggttaattccctttttaggggcttaccatctttactttctttagtagttacaatattaaagtagtcttgtaacctatcccagttattcttcattagatctacctcctatgcttacattatacatatattgtactgatatgtcaaagtccaggcattaactgatatctgatatgcctatatttttaccccatatcagtctgatatcccacatatcagttgaaactacaaaatcacaaaggcattggtatcactggcgtagagggatatcagttatgccccctttatatatacatagtattatatatactatataataatatattattatatatagtatatatatatattacatggtgattacatcaatggcaggctattgccttgcctccattatcattacggcaggcatatccatgcttccgagcttttgccctatatagaaaaacccagacggtcagc